European Patent Application EP 4 700 127 A1, published February 25, 2026. Title: 一种制备基因编辑鸡的方法. Applicant: 中国农业大学. The sequence listing filed with the application follows.

SEQUENCE LISTING (37 sequences)

SEQ ID NO: 1 - DNA, 20 bp, synthetic construct
  source 1..20: mol_type = other DNA
tacctgggtcatgagccggt

SEQ ID NO: 2 - DNA, 20 bp, synthetic construct
  source 1..20: mol_type = other DNA
cggcggcaataaatagcgaa

SEQ ID NO: 3 - DNA, 20 bp, synthetic construct
  source 1..20: mol_type = other DNA
gcgagcgggatgagcttgcg

SEQ ID NO: 4 - DNA, 405 bp, synthetic construct
  source 1..405: mol_type = other DNA
atcggaagacctcaccgcggcggcaataaatagcgaagttttagagctagaaatagcaagttaaaataaggctagtccgttatcaacttgaaaaagtggcaccgagtcggtgcttttttgagggcctatttcccatgattccttcatatttgcatatacgatacaaggctgttagagagataattggaattaatttgactgtaaacacaaagatattagtacaaaatacgtgacgtagaaagtaataatttcttgggtagtttgcagttttaaaattatgttttaaaatggactatcatatgcttaccgtaacttgaaagtatttcgatttcttggctttatatatcttgtggaaaggacgaaacaccgtacctgggtcatgagccggtgtttgggtcttcatcg

SEQ ID NO: 5 - DNA, 404 bp, synthetic construct
  source 1..404: mol_type = other DNA
atcggaagacctcaccgcgagcgggatgagcttgcggttttagagctagaaatagcaagttaaaataaggctagtccgttatcaacttgaaaaagtggcaccgagtcggtgcttttttgagggcctatttcccatgattccttcatatttgcatatacgatacaaggctgttagagagataattggaattaatttgactgtaaacacaaagatattagtacaaaatacgtgacgtagaaagtaataatttcttgggtagtttgcagttttaaaattatgttttaaaatggactatcatatgcttaccgtaacttgaaagtatttcgatttcttggctttatatatcttgtggaaaggacgaaacaccgtacctgggtcatgagccggtgtttgggtcttcatcg

SEQ ID NO: 6 - DNA, 56 bp, synthetic construct
  source 1..56: mol_type = other DNA
atcggaagacctcaccgcggcggcaataaatagcgaagttttagagctagaaatag

SEQ ID NO: 7 - DNA, 54 bp, synthetic construct
  source 1..54: mol_type = other DNA
cgatgaagacccaaacaccggctcatgacccaggtacggtgtttcgtcctttcc

SEQ ID NO: 8 - DNA, 55 bp, synthetic construct
  source 1..55: mol_type = other DNA
atcggaagacctcaccgcgagcgggatgagcttgcggttttagagctagaaatag

SEQ ID NO: 9 - DNA, 18 bp, synthetic construct
  source 1..18: mol_type = other DNA
aatttcccctctcactcc

SEQ ID NO: 10 - DNA, 18 bp, synthetic construct
  source 1..18: mol_type = other DNA
ctttgccatcctactctg

SEQ ID NO: 11 - DNA, 40 bp, synthetic construct
  source 1..40: mol_type = other DNA
taatacgactcactatagggtacctgggtcatgagccggt

SEQ ID NO: 12 - DNA, 40 bp, synthetic construct
  source 1..40: mol_type = other DNA
taatacgactcactataggggcgagcgggatgagcttgcg

SEQ ID NO: 13 - DNA, 24 bp, synthetic construct
  source 1..24: mol_type = other DNA
aaaaaagcaccgactcggtgccac

SEQ ID NO: 14 - DNA, 20 bp, synthetic construct
  source 1..20: mol_type = other DNA
taatacgactcactataggg

SEQ ID NO: 15 - DNA, 18 bp, synthetic construct
  source 1..18: mol_type = other DNA
gcaccgactcggtgccac

SEQ ID NO: 16 - DNA, 41 bp, synthetic construct
  source 1..41: mol_type = other DNA
caagcgcatgctggccagcgccggcgagctgcagaagggca

SEQ ID NO: 17 - DNA, 38 bp, synthetic construct
  source 1..38: mol_type = other DNA
tctcgtacagaccggtgatgctctggtggatcagggtg

SEQ ID NO: 18 - DNA, 160 bp, synthetic construct
  source 1..160: mol_type = other DNA
catcaccggtctgtacgagacccgcatcgacctgagccagctgggcggcgacggcggctccggacctccaaagaaaaagagaaaagtagaggacccaaagaaaaagagaaaagtatacccctacgacgtgcccgactacgcctgttaactcgagcaccac

SEQ ID NO: 19 - DNA, 35 bp, synthetic construct
  source 1..35: mol_type = other DNA
catcaccggtctgtacgagacccgcatcgacctga

SEQ ID NO: 20 - DNA, 43 bp, synthetic construct
  source 1..43: mol_type = other DNA
cagtggtggtggtggtggtgctcgagttaacaggcgtagtcgg

SEQ ID NO: 21 - DNA, 18 bp, synthetic construct
  source 1..18: mol_type = other DNA
gcccttcgctatttattg

SEQ ID NO: 22 - DNA, 18 bp, synthetic construct
  source 1..18: mol_type = other DNA
cgtgagctccttgaagcg

SEQ ID NO: 23 - DNA, 22 bp, synthetic construct
  source 1..22: mol_type = other DNA
gcccttcgctatttattgccgc

SEQ ID NO: 24 - DNA, 23 bp, synthetic construct
  source 1..23: mol_type = other DNA
ggataaactcgctgctctgccca

SEQ ID NO: 25 - DNA, 22 bp, synthetic construct
  source 1..22: mol_type = other DNA
cctgagcgaactggataaggcc

SEQ ID NO: 26 - DNA, 22 bp, synthetic construct
  source 1..22: mol_type = other DNA
ctcttggcgatcatcttccgca

SEQ ID NO: 27 - DNA, 21 bp, synthetic construct
  source 1..21: mol_type = other DNA
gctcatcccgctcgcctacaa

SEQ ID NO: 28 - DNA, 23 bp, synthetic construct
  source 1..23: mol_type = other DNA
atctcttcaatttcccctctcac

SEQ ID NO: 29 - DNA, 23 bp, synthetic construct
  source 1..23: mol_type = other DNA
gcacccgctcagcagcagcagca

SEQ ID NO: 30 - DNA, 193 bp, synthetic construct
  source 1..193: mol_type = other DNA
cagccatatgcccaagaaaaagcgcaaagtgggtggcagcccgaagaagaagcgcaaagtgggcggcagtccgaaaaagaaacgcaaagtgggcggtagcccgaagaagaagcgcaaagtgggtatccacggtgtcccagcagccaccatggacaagaagtacagcatcggcctggacatcggtaccaacagc

SEQ ID NO: 31 - DNA, 29 bp, synthetic construct
  source 1..29: mol_type = other DNA
ggaattccatatgcccaagaaaaagcgca

SEQ ID NO: 32 - DNA, 23 bp, synthetic construct
  source 1..23: mol_type = other DNA
cggggtaccgatgtccaggccga

SEQ ID NO: 33 - DNA, 58 bp, synthetic construct
  source 1..58: mol_type = other DNA
gtcgtaggggtatacttttctctttttctttgggtcctctacttttctctttttcttt

SEQ ID NO: 34 - protein, 5 aa, synthetic construct
GGGGS

SEQ ID NO: 35 - DNA, 759 bp, synthetic construct
  source 1..759: mol_type = other DNA
ggtggtggcggtagcggcggcggcggtagtatggtcagcaaaggcgaagaggacaacatggcaagtctgccggcaacccacgaactgcatatttttggcagcatcaacggcgtcgacttcgatatggtaggtcaaggtaccggtaatccgaacgacggttacgaagagctgaacctgaagagcaccaaaggcgatctgcaatttagtccgtggattctggttccgcacattggttacggcttccatcagtatctgccgtatccggacggtatgagtccgtttcaggcagcgatggtagatggttctggttatcaggtccatcgtaccatgcagtttgaagacggcgcaagtctgaccgttaactatcgctacacctacgaaggcagccatatcaaaggcgaagcgcaggttaaaggtaccggttttccggctgacggtccggttatgaccaatagtctgaccgctgctgattggtgtcgtagcaaaaagacctacccgaacgacaagaccatcatctccaccttcaagtggagctacaccaccggtaacggtaaacgctatcgtagtaccgcacgtaccacctatacctttgctaaaccgatggcggcgaactatctgaaaaaccaaccgatgtacgtcttccgcaagaccgaactgaagcacagcaaaaccgagctgaacttcaaagaatggcagaaagcgttcaccgacgttatgggtatggacgaactgtacaagccgaagaagaagcgcaaagtg

SEQ ID NO: 36 - DNA, 59 bp, synthetic construct
  source 1..59: mol_type = other DNA
gaaaagtatacccctacgacgtgcccgactacgcctgtggtggtggcggtagcggcggc

SEQ ID NO: 37 - DNA, 59 bp, synthetic construct
  source 1..59: mol_type = other DNA
ggtggtggtggtggtgctcgagcactttgcgcttcttcttcggcttgtacagttcgtcc